European Patent Application EP 4 600 258 A1, published August 13, 2025. Title: KERATIN YK93-6, PREPARATION METHOD THEREFOR, PHARMACEUTICAL COMPOSITION THEREOF, AND USE THEREOF. Applicant: Institute of Materia Medica Chinese Academy Of Medical Sciences. The sequence listing filed with the application follows.

SEQUENCE LISTING (2 sequences)

SEQ ID NO: 1 - protein, 466 aa, Manis pentadactyla
MATQICSPVFSSGSVKGLCGTAGSLSRVTSVRSLGSCRVPSLAGAVGSASSIRLGLSGFGSCLPGPYLSTGCYPSGFGSGGLFFEGAFNGSEKETMQFLNDRLASYLEKVRQLERENAELERRIREWYEAQIPYICPDYQSYYKTIEELQQKILLTKAENARLVLQIDNAKLAADDFRTKYETELGLRQLVEADINGLRRILDELTLCRADLEMQVESLKEELLCLKKNHEEEVNVLRGQLGDRLNVEVDAAPTVDLNKILDDMRCQYETLVENNRRDVEAWFNTQTEELNQQVVSSSEQLQSCQTDIIELRRTVNALEIELQAQHSMRSSLESTLTETEARYSSQLSQLQFMITNVESQLAEIRCDLERQNQEYQVLLDVKARLESEIATYRRLLEGEDSKLPPHPCATECKPAIRVPYIPAVPCGPTVPCAPGPQISTQIRTITEEIRDGKVISSREHLQPCPL

SEQ ID NO: 2 - DNA, 1398 bp, Manis pentadactyla
  source 1..1398: mol_type = genomic DNA
atggcaacccagatttgtagcccggtttttagtagtggtagcgtgaaaggcctgtgcggtaccgcaggcagcctgagtcgtgttaccagtgtgcgtagtctgggtagctgtcgtgtgccgagtctggccggtgcagtgggcagcgctagtagtattcgcctgggtctgagtggctttggcagctgtctgccgggcccgtatctgagtaccggttgttatccgagcggttttggcagcggtggcctgtttttcgaaggtgcattcaatggcagcgaaaaagaaaccatgcagtttctgaatgatcgtctggccagttatctggaaaaagtgcgccagctggaacgcgaaaatgccgaactggaacgccgcattcgtgaatggtatgaagcccagattccgtatatttgtccggattatcagagttattacaaaaccattgaggaactgcagcagaaaattctgctgaccaaagcagaaaatgcacgcctggtgctgcagattgataatgcaaaactggccgcagatgattttcgtaccaaatatgaaaccgaactgggcctgcgtcagctggttgaagcagatattaatggcctgcgtcgcattctggatgaactgaccctgtgccgcgccgatctggaaatgcaggtggaaagtctgaaagaagaactgctgtgtctgaaaaagaatcatgaagaagaagttaacgtgctgcgcggccagctgggcgatcgtctgaatgttgaagtggatgcagcaccgaccgtggatctgaataagattctggatgatatgcgctgtcagtatgaaaccctggtggaaaataatcgtcgcgatgttgaagcctggtttaatacccagaccgaagaactgaatcagcaggttgtgagcagtagcgaacagctgcagagctgtcagaccgatattattgaactgcgtcgtaccgttaatgcactggaaattgaactgcaggcacagcatagcatgcgtagcagcctggaaagtaccctgaccgaaaccgaagcccgctatagtagccagctgagtcagctgcagtttatgattaccaatgttgaaagccagctggcagaaattcgctgtgatctggaacgtcagaatcaggaatatcaggttctgctggatgttaaagcccgtctggaaagtgaaattgcaacctatcgccgcctgctggaaggtgaagatagtaaactgccgccgcatccgtgtgcaaccgaatgtaaaccggcaattcgcgtgccgtatattccggccgttccgtgcggtccgaccgtgccttgtgcaccgggtccgcagattagcacccagattcgcaccattaccgaagaaattcgcgatggtaaagtgattagtagccgtgaacatctgcagccgtgcccgctg